European Patent Application EP 4 501 967 A1, published February 5, 2025. Title: pH-dependent anti-sulfated glycosaminoglycan antibodies and antibody -drug conjugates. Applicant: The Univeristy of Tokyo. The sequence listing filed with the application follows.

SEQUENCE LISTING (50 sequences)

SEQ ID NO: 1 - protein, 8 aa, synthetic construct
  REGION 1..8: note = Amino acid sequence of CDR1 of heavy chain of antibody 1 and antibody 4
GGFITSHH

SEQ ID NO: 2 - protein, 7 aa, synthetic construct
  REGION 1..7: note = Amino acid sequence of CDR2 of heavy chain of antibody 1 and antibody 4
LHHTGTT

SEQ ID NO: 3 - protein, 16 aa, synthetic construct
  REGION 1..16: note = Amino acid sequence of CDR3 of heavy chain of antibody 1 and antibody 4
VREDSSSWHPGRYIQL

SEQ ID NO: 4 - protein, 11 aa, synthetic construct
  REGION 1..11: note = Amino acid sequence of CDR1 of light chain of antibody 1 and antibody 4
QSLLQNNRYNR

SEQ ID NO: 5 - skipped

SEQ ID NO: 6 - protein, 9 aa, synthetic construct
  REGION 1..9: note = Amino acid sequence of CDR3 of light chain of antibody 1 and antibody 4
MHALEPPYT

SEQ ID NO: 7 - protein, 8 aa, synthetic construct
  REGION 1..8: note = Amino acid sequence of CDR1 of heavy chain of antibody 2
GFTFNTYT

SEQ ID NO: 8 - protein, 8 aa, synthetic construct
  REGION 1..8: note = Amino acid sequence of CDR2 of heavy chain of antibody 2
ISLSSNTI

SEQ ID NO: 9 - protein, 18 aa, synthetic construct
  REGION 1..18: note = Amino acid sequence of CDR3 of heavy chain of antibody 2
ARAESYYDSHYYYNGLDV

SEQ ID NO: 10 - protein, 7 aa, synthetic construct
  REGION 1..7: note = Amino acid sequence of CDR1 of light chain of antibody 2
QSVGGRY

SEQ ID NO: 11 - skipped

SEQ ID NO: 12 - protein, 9 aa, synthetic construct
  REGION 1..9: note = Amino acid sequence of CDR3 of light chain of antibody 2
QQYGSSPRT

SEQ ID NO: 13 - protein, 8 aa, synthetic construct
  REGION 1..8: note = Amino acid sequence of CDR1 of heavy chain of antibody 3
GFTFSDYY

SEQ ID NO: 14 - protein, 8 aa, synthetic construct
  REGION 1..8: note = Amino acid sequence of CDR2 of heavy chain of antibody 3
ISISGTTR

SEQ ID NO: 15 - protein, 19 aa, synthetic construct
  REGION 1..19: note = Amino acid sequence of CDR3 of heavy chain of antibody 3
ARGPELLSQNYYYYYGMDV

SEQ ID NO: 16 - protein, 12 aa, synthetic construct
  REGION 1..12: note = Amino acid sequence of CDR1 of light chain of antibody 3
ETLLYRSNNKNY

SEQ ID NO: 17 - skipped

SEQ ID NO: 18 - protein, 9 aa, synthetic construct
  REGION 1..9: note = Amino acid sequence of CDR3 of light chain of antibody 3
QQYYTTPRT

SEQ ID NO: 19 - DNA, 366 bp, synthetic construct
  misc_feature 1..366: note = Nucleotide sequence of cDNA encoding the variable region of the heavy chain of antibody 1
  source 1..366: mol_type = other DNA
caggtgcagttacaagagagcggccccggcctggtgaagcccagcgagaccctgtccctgacctgcaccgtgtccggcggcttcatcacctcccaccactggagctggatcagacagccccccggccagggcctggagtggatcggcttcctgcaccacaccggcaccacccactacaacccctccctgaagtccagagtgaccacctccgtggacaccgccaagaaccagttcagcctgaccctgaagagcctgaccgccgccgacaccgccgtgtactactgcgtgagggaggactccagcagctggcaccccggcagatacatccagctgtggggccagggcaccctggtgaccgtgagcgcc

SEQ ID NO: 20 - protein, 122 aa, synthetic construct
  REGION 1..122: note = Amino acid sequence of the variable region of the heavy chain of antibody 1
QVQLQESGPGLVKPSETLSLTCTVSGGFITSHHWSWIRQPPGQGLEWIGFLHHTGTTHYNPSLKSRVTTSVDTAKNQFSLTLKSLTAADTAVYYCVREDSSSWHPGRYIQLWGQGTLVTVSA

SEQ ID NO: 21 - DNA, 336 bp, synthetic construct
  misc_feature 1..336: note = Nucleotide sequence of cDNA encoding the variable region of the light chain of antibody 1
  source 1..336: mol_type = other DNA
gacgtagtgatgacccagagccccctgagcctgcccgtgacccccggcgagcccgccagcatcagttgcagaagcagccagagcctgcttcaaaacaacagatacaacagattcgactggtatctccaaaagcccggccagagccccagaatcctgatctacctgggcagcaacagagccagcggcgtgcccgacagattcagcggcaccaccagcggcaccgactacaccctgagaatcagcagagtggaggccgaggacgccggcgtgtactactgtatgcacgccctggagcccccctacaccttcggccagggcaccaagctggagatcaag

SEQ ID NO: 22 - protein, 112 aa, synthetic construct
  REGION 1..112: note = Amino acid sequence of the variable region of the light chain of antibody 1
DVVMTQSPLSLPVTPGEPASISCRSSQSLLQNNRYNRFDWYLQKPGQSPRILIYLGSNRASGVPDRFSGTTSGTDYTLRISRVEAEDAGVYYCMHALEPPYTFGQGTKLEIK

SEQ ID NO: 23 - DNA, 375 bp, synthetic construct
  misc_feature 1..375: note = Nucleotide sequence of cDNA encoding the variable region of the heavy chain of antibody 2
  source 1..375: mol_type = other DNA
gaggtgcagctggtggagagcggcggcggcctggtgcagcccggcggcagcctgagactgagctgcgccgccagcggcttcacattcaacacctacaccatgaactgggtgagacaggcccccggcaagggcctggagtgggtggcctacatcagcctgagcagcaacaccatcttctacgccccttccgtgaagggccggtttacagtgtcccgggataatgccaagaattccctgtacctgcagatgaatacactgtccgatgatgacacagccgtgtactactgtgcccgcgccgagagctactacgactcccactactactacaacggcctggacgtgtggggccagggcaccaccgtgtccgtgacatcc

SEQ ID NO: 24 - protein, 125 aa, synthetic construct
  REGION 1..125: note = Amino acid sequence of the variable region of the heavy chain of antibody 2
EVQLVESGGGLVQPGGSLRLSCAASGFTFNTYTMNWVRQAPGKGLEWVAYISLSSNTIFYAPSVKGRFTVSRDNAKNSLYLQMNTLSDDDTAVYYCARAESYYDSHYYYNGLDVWGQGTTVSVTS

SEQ ID NO: 25 - DNA, 324 bp, synthetic construct
  misc_feature 1..324: note = Nucleotide sequence of cDNA encoding the variable region of the light chain of antibody 2
  source 1..324: mol_type = other DNA
gaaatcgtgctgacacagtccccaggcacactgtccctgtccccaggcgagcgcgccaccctgagctgtagagccagccagtccgtgggcggcaggtacctggcctggtaccagaagaaggccggccaggcccctaggctgctgatctccgccgccagcagcagagccacaggcatccctgatcgcttttccggctccggctccggcacagattttacactgaccatcagcagggtggagcccgaggacttcgccgtgtactactgccagcagtacggcagcagccccagaaccttcggccagggcaccaaggtggagatcaag

SEQ ID NO: 26 - protein, 108 aa, synthetic construct
  REGION 1..108: note = Amino acid sequence of the variable region of the light chain of antibody 2
EIVLTQSPGTLSLSPGERATLSCRASQSVGGRYLAWYQKKAGQAPRLLISAASSRATGIPDRFSGSGSGTDFTLTISRVEPEDFAVYYCQQYGSSPRTFGQGTKVEIK

SEQ ID NO: 27 - DNA, 378 bp, synthetic construct
  misc_feature 1..378: note = Nucleotide sequence of cDNA encoding the variable region of the heavy chain of antibody 3
  source 1..378: mol_type = other DNA
caggtgcagctggtggagtccggcggcggcctggtgaagcccggcggcagcctgagactgagctgtgccgccagcggctttacattttccgattactacatgtcctggatccgccaggccccaggcaagggcctggagtgggtgagctacatctccatctccggcacaacacgctactacgccgattccgtgaagggccggttcacaatctcccgggataatgccaagaattccctgagcctgcagatgaacagcctgagggccgaggacaccgccgtgtactactgcgccaggggccccgagctgctgagccagaactactactactactacggcatggacgtgtggggccagggcaccaccgtgaccgtgagcctg

SEQ ID NO: 28 - protein, 126 aa, synthetic construct
  REGION 1..126: note = Amino acid sequence of the variable region of the heavy chain of antibody 3
QVQLVESGGGLVKPGGSLRLSCAASGFTFSDYYMSWIRQAPGKGLEWVSYISISGTTRYYADSVKGRFTISRDNAKNSLSLQMNSLRAEDTAVYYCARGPELLSQNYYYYYGMDVWGQGTTVTVSL

SEQ ID NO: 29 - DNA, 339 bp, synthetic construct
  misc_feature 1..339: note = Nucleotide sequence of cDNA encoding the variable region of the light chain of antibody 3
  source 1..339: mol_type = other DNA
gacatcgagatgacccagagccccgacagcctggccgtgagcctgggcgagagagccaccatcaactgcaagagcagcgagaccctgctgtacagaagcaacaacaagaattacctggcctggtaccagcagaagcccggccagccccctaggctgctgctgtactgggccagcacacgggagtccggcgtgcctgacaggatctccggctccggctccggcaccgatttcaccctgaccatctcctccctgcaggccgaggatgtggccgtgtactactgccagcagtactacaccacaccacggacattcggccagggcacaaaggtggagatcaag

SEQ ID NO: 30 - protein, 113 aa, synthetic construct
  REGION 1..113: note = Amino acid sequence of the variable region of the light chain of antibody 3
DIEMTQSPDSLAVSLGERATINCKSSETLLYRSNNKNYLAWYQQKPGQPPRLLLYWASTRESGVPDRISGSGSGTDFTLTISSLQAEDVAVYYCQQYYTTPRTFGQGTKVEIK

SEQ ID NO: 31 - DNA, 360 bp, synthetic construct
  misc_feature 1..360: note = Nucleotide sequence of cDNA encoding the variable region of the heavy chain of antibody 4
  source 1..360: mol_type = other DNA
gaggtgcagctggttgaatctggcggcggattggttcagcctggcggatctctgagactgtcttgtgctgcctctggcggcttcatcacctctcaccattgggtccgacaggcccctggcaaaggactggaatgggttgccagactgcaccacaccggcaccacacactacgccgattctgtgaagggcagattcaccatctccgccgacacctccaagaacaccgcctacctgcagatgaactccctgagagccgaggacaccgccgtgtactactgtgtgcgcgaggactcctcttcttggcaccctggcagatatatccagctgtggggccagggcacactggtcacagtttcttcc

SEQ ID NO: 32 - protein, 120 aa, synthetic construct
  REGION 1..120: note = Amino acid sequence of the variable region of the heavy chain of antibody 4
EVQLVESGGGLVQPGGSLRLSCAASGGFITSHHWVRQAPGKGLEWVARLHHTGTTHYADSVKGRFTISADTSKNTAYLQMNSLRAEDTAVYYCVREDSSSWHPGRYIQLWGQGTLVTVSS

SEQ ID NO: 33 - DNA, 336 bp, synthetic construct
  misc_feature 1..336: note = Nucleotide sequence of cDNA encoding the variable region of the light chain of antibody 4
  source 1..336: mol_type = other DNA
gacatccagatgacccagtctccatcctctctgtccgcctctgtgggcgacagagtgaccatctcctgccggtcatctcagtccctgctgcagaacaaccggtacaacagattcgactggtatcagcagaagcccggcaaggcccctaagctgctgatctacctgggctccaatagagcctctggcgtgccctctagattctccggctctagatctggcaccgactttaccctgacaatctccagcctgcagcctgaggacttcgccacctactactgcatgcacgccctggaacctccatacacctttggccagggcaccaaggtggaaatcaag

SEQ ID NO: 34 - protein, 112 aa, synthetic construct
  REGION 1..112: note = Amino acid sequence of the variable region of the light chain of antibody 4
DIQMTQSPSSLSASVGDRVTISCRSSQSLLQNNRYNRFDWYQQKPGKAPKLLIYLGSNRASGVPSRFSGSRSGTDFTLTISSLQPEDFATYYCMHALEPPYTFGQGTKVEIK

SEQ ID NO: 35 - DNA, 1356 bp, synthetic construct
  misc_feature 1..1356: note = Nucleotide sequence of the heavy chain of antibody 1
  source 1..1356: mol_type = other DNA
caggtgcagttacaagagagcggccccggcctggtgaagcccagcgagaccctgtccctgacctgcaccgtgtccggcggcttcatcacctcccaccactggagctggatcagacagccccccggccagggcctggagtggatcggcttcctgcaccacaccggcaccacccactacaacccctccctgaagtccagagtgaccacctccgtggacaccgccaagaaccagttcagcctgaccctgaagagcctgaccgccgccgacaccgccgtgtactactgcgtgagggaggactccagcagctggcaccccggcagatacatccagctgtggggccagggcaccctggtgaccgtgagcgccgctagcaccaagggcccatcggtcttccccctggcaccctcctccaagagcacctctgggggcacagcggccctgggctgcctggtcaaggactacttccccgaaccggtgacggtgtcgtggaactcaggcgccctgaccagcggcgtgcacaccttcccggctgtcctacagtcctcaggactctactccctcagcagcgtggtgaccgtgccctccagcagcttgggcacccagacctacatctgcaacgtgaatcacaagcccagcaacaccaaggtggacaagaaagttgagcccaaatcttgtgacaaaactcacacatgcccaccgtgcccagcacctgaactcctggggggaccgtcagtcttcctcttccccccaaaacccaaggacaccctcatgatctcccggacccctgaggtcacgtgcgtggtggtggacgtgagccacgaagaccccgaggtcaagttcaactggtacgtggacggcgtggaggtgcataatgccaagacaaagccgcgggaggagcagtacaacagcacgtaccgtgtggtcagcgtcctcaccgtcctgcaccaggactggctgaatggcaaggagtacaagtgcaaggtctccaacaaagccctcccagcccccatcgagaaaaccatctccaaagccaaagggcagccccgagaaccacaggtgtacaccctgcccccatcccgggatgagctgaccaagaaccaggtcagcctgacctgcctggtcaaaggcttctatcccagcgacatcgccgtggagtgggagagcaatgggcagccggagaacaactacaagaccacgcctcccgtgctggactccgacggctccttcttcctctacagcaagctcaccgtggacaagagcaggtggcagcaggggaacgtcttctcatgctccgtgatgcatgaggctctgcacaaccactacacgcagaagagcctctccctgtctccgggtaaa

SEQ ID NO: 36 - protein, 452 aa, synthetic construct
  REGION 1..452: note = Amino acid sequence of heavy chain of antibody 1
QVQLQESGPGLVKPSETLSLTCTVSGGFITSHHWSWIRQPPGQGLEWIGFLHHTGTTHYNPSLKSRVTTSVDTAKNQFSLTLKSLTAADTAVYYCVREDSSSWHPGRYIQLWGQGTLVTVSAASTKGPSVFPLAPSSKSTSGGTAALGCLVKDYFPEPVTVSWNSGALTSGVHTFPAVLQSSGLYSLSSVVTVPSSSLGTQTYICNVNHKPSNTKVDKKVEPKSCDKTHTCPPCPAPELLGGPSVFLFPPKPKDTLMISRTPEVTCVVVDVSHEDPEVKFNWYVDGVEVHNAKTKPREEQYNSTYRVVSVLTVLHQDWLNGKEYKCKVSNKALPAPIEKTISKAKGQPREPQVYTLPPSRDELTKNQVSLTCLVKGFYPSDIAVEWESNGQPENNYKTTPPVLDSDGSFFLYSKLTVDKSRWQQGNVFSCSVMHEALHNHYTQKSLSLSPGK

SEQ ID NO: 37 - DNA, 657 bp, synthetic construct
  misc_feature 1..657: note = Nucleotide sequence of the light chain of antibody 1
  source 1..657: mol_type = other DNA
gacgtagtgatgacccagagccccctgagcctgcccgtgacccccggcgagcccgccagcatcagttgcagaagcagccagagcctgcttcaaaacaacagatacaacagattcgactggtatctccaaaagcccggccagagccccagaatcctgatctacctgggcagcaacagagccagcggcgtgcccgacagattcagcggcaccaccagcggcaccgactacaccctgagaatcagcagagtggaggccgaggacgccggcgtgtactactgtatgcacgccctggagcccccctacaccttcggccagggcaccaagctggagatcaagcgtacggtggctgcaccatctgtcttcatcttcccgccatctgatgagcagttgaaatctggaactgcctctgttgtgtgcctgctgaataacttctatcccagagaggccaaagtacagtggaaggtggataacgccctccaatcgggtaactcccaggagagtgtcacagagcaggacagcaaggacagcacctacagcctcagcagcaccctgacgctgagcaaagcagactacgagaaacacaaagtctacgcctgcgaagtcacccatcagggcctgagctcgcccgtcacaaagagcttcaacaggggagagtgt

SEQ ID NO: 38 - protein, 219 aa, synthetic construct
  REGION 1..219: note = Amino acid sequence of the light chain of antibody 1
DVVMTQSPLSLPVTPGEPASISCRSSQSLLQNNRYNRFDWYLQKPGQSPRILIYLGSNRASGVPDRFSGTTSGTDYTLRISRVEAEDAGVYYCMHALEPPYTFGQGTKLEIKRTVAAPSVFIFPPSDEQLKSGTASVVCLLNNFYPREAKVQWKVDNALQSGNSQESVTEQDSKDSTYSLSSTLTLSKADYEKHKVYACEVTHQGLSSPVTKSFNRGEC

SEQ ID NO: 39 - DNA, 1365 bp, synthetic construct
  misc_feature 1..1365: note = Nucleotide sequence of the heavy chain of antibody 2
  source 1..1365: mol_type = other DNA
gaggtgcagctggtggagagcggcggcggcctggtgcagcccggcggcagcctgagactgagctgcgccgccagcggcttcacattcaacacctacaccatgaactgggtgagacaggcccccggcaagggcctggagtgggtggcctacatcagcctgagcagcaacaccatcttctacgccccttccgtgaagggccggtttacagtgtcccgggataatgccaagaattccctgtacctgcagatgaatacactgtccgatgatgacacagccgtgtactactgtgcccgcgccgagagctactacgactcccactactactacaacggcctggacgtgtggggccagggcaccaccgtgtccgtgacatccgctagcaccaagggcccatcggtcttccccctggcaccctcctccaagagcacctctgggggcacagcggccctgggctgcctggtcaaggactacttccccgaaccggtgacggtgtcgtggaactcaggcgccctgaccagcggcgtgcacaccttcccggctgtcctacagtcctcaggactctactccctcagcagcgtggtgaccgtgccctccagcagcttgggcacccagacctacatctgcaacgtgaatcacaagcccagcaacaccaaggtggacaagaaagttgagcccaaatcttgtgacaaaactcacacatgcccaccgtgcccagcacctgaactcctggggggaccgtcagtcttcctcttccccccaaaacccaaggacaccctcatgatctcccggacccctgaggtcacgtgcgtggtggtggacgtgagccacgaagaccccgaggtcaagttcaactggtacgtggacggcgtggaggtgcataatgccaagacaaagccgcgggaggagcagtacaacagcacgtaccgtgtggtcagcgtcctcaccgtcctgcaccaggactggctgaatggcaaggagtacaagtgcaaggtctccaacaaagccctcccagcccccatcgagaaaaccatctccaaagccaaagggcagccccgagaaccacaggtgtacaccctgcccccatcccgggatgagctgaccaagaaccaggtcagcctgacctgcctggtcaaaggcttctatcccagcgacatcgccgtggagtgggagagcaatgggcagccggagaacaactacaagaccacgcctcccgtgctggactccgacggctccttcttcctctacagcaagctcaccgtggacaagagcaggtggcagcaggggaacgtcttctcatgctccgtgatgcatgaggctctgcacaaccactacacgcagaagagcctctccctgtctccgggtaaa

SEQ ID NO: 40 - protein, 455 aa, synthetic construct
  REGION 1..455: note = Amino acid sequence of heavy chain of antibody 2
EVQLVESGGGLVQPGGSLRLSCAASGFTFNTYTMNWVRQAPGKGLEWVAYISLSSNTIFYAPSVKGRFTVSRDNAKNSLYLQMNTLSDDDTAVYYCARAESYYDSHYYYNGLDVWGQGTTVSVTSASTKGPSVFPLAPSSKSTSGGTAALGCLVKDYFPEPVTVSWNSGALTSGVHTFPAVLQSSGLYSLSSVVTVPSSSLGTQTYICNVNHKPSNTKVDKKVEPKSCDKTHTCPPCPAPELLGGPSVFLFPPKPKDTLMISRTPEVTCVVVDVSHEDPEVKFNWYVDGVEVHNAKTKPREEQYNSTYRVVSVLTVLHQDWLNGKEYKCKVSNKALPAPIEKTISKAKGQPREPQVYTLPPSRDELTKNQVSLTCLVKGFYPSDIAVEWESNGQPENNYKTTPPVLDSDGSFFLYSKLTVDKSRWQQGNVFSCSVMHEALHNHYTQKSLSLSPGK

SEQ ID NO: 41 - DNA, 645 bp, synthetic construct
  misc_feature 1..645: note = Nucleotide sequence of the light chain of antibody 2
  source 1..645: mol_type = other DNA
gaaatcgtgctgacacagtccccaggcacactgtccctgtccccaggcgagcgcgccaccctgagctgtagagccagccagtccgtgggcggcaggtacctggcctggtaccagaagaaggccggccaggcccctaggctgctgatctccgccgccagcagcagagccacaggcatccctgatcgcttttccggctccggctccggcacagattttacactgaccatcagcagggtggagcccgaggacttcgccgtgtactactgccagcagtacggcagcagccccagaaccttcggccagggcaccaaggtggagatcaagcgtacggtggctgcaccatctgtcttcatcttcccgccatctgatgagcagttgaaatctggaactgcctctgttgtgtgcctgctgaataacttctatcccagagaggccaaagtacagtggaaggtggataacgccctccaatcgggtaactcccaggagagtgtcacagagcaggacagcaaggacagcacctacagcctcagcagcaccctgacgctgagcaaagcagactacgagaaacacaaagtctacgcctgcgaagtcacccatcagggcctgagctcgcccgtcacaaagagcttcaacaggggagagtgt

SEQ ID NO: 42 - protein, 215 aa, synthetic construct
  REGION 1..215: note = Amino acid sequence of the light chain of antibody 2
EIVLTQSPGTLSLSPGERATLSCRASQSVGGRYLAWYQKKAGQAPRLLISAASSRATGIPDRFSGSGSGTDFTLTISRVEPEDFAVYYCQQYGSSPRTFGQGTKVEIKRTVAAPSVFIFPPSDEQLKSGTASVVCLLNNFYPREAKVQWKVDNALQSGNSQESVTEQDSKDSTYSLSSTLTLSKADYEKHKVYACEVTHQGLSSPVTKSFNRGEC

SEQ ID NO: 43 - DNA, 1368 bp, synthetic construct
  misc_feature 1..1368: note = Nucleotide sequence of the heavy chain of antibody 3
  source 1..1368: mol_type = other DNA
caggtgcagctggtggagtccggcggcggcctggtgaagcccggcggcagcctgagactgagctgtgccgccagcggctttacattttccgattactacatgtcctggatccgccaggccccaggcaagggcctggagtgggtgagctacatctccatctccggcacaacacgctactacgccgattccgtgaagggccggttcacaatctcccgggataatgccaagaattccctgagcctgcagatgaacagcctgagggccgaggacaccgccgtgtactactgcgccaggggccccgagctgctgagccagaactactactactactacggcatggacgtgtggggccagggcaccaccgtgaccgtgagcctggctagcaccaagggcccatcggtcttccccctggcaccctcctccaagagcacctctgggggcacagcggccctgggctgcctggtcaaggactacttccccgaaccggtgacggtgtcgtggaactcaggcgccctgaccagcggcgtgcacaccttcccggctgtcctacagtcctcaggactctactccctcagcagcgtggtgaccgtgccctccagcagcttgggcacccagacctacatctgcaacgtgaatcacaagcccagcaacaccaaggtggacaagaaagttgagcccaaatcttgtgacaaaactcacacatgcccaccgtgcccagcacctgaactcctggggggaccgtcagtcttcctcttccccccaaaacccaaggacaccctcatgatctcccggacccctgaggtcacgtgcgtggtggtggacgtgagccacgaagaccccgaggtcaagttcaactggtacgtggacggcgtggaggtgcataatgccaagacaaagccgcgggaggagcagtacaacagcacgtaccgtgtggtcagcgtcctcaccgtcctgcaccaggactggctgaatggcaaggagtacaagtgcaaggtctccaacaaagccctcccagcccccatcgagaaaaccatctccaaagccaaagggcagccccgagaaccacaggtgtacaccctgcccccatcccgggatgagctgaccaagaaccaggtcagcctgacctgcctggtcaaaggcttctatcccagcgacatcgccgtggagtgggagagcaatgggcagccggagaacaactacaagaccacgcctcccgtgctggactccgacggctccttcttcctctacagcaagctcaccgtggacaagagcaggtggcagcaggggaacgtcttctcatgctccgtgatgcatgaggctctgcacaaccactacacgcagaagagcctctccctgtctccgggtaaa

SEQ ID NO: 44 - protein, 456 aa, synthetic construct
  REGION 1..456: note = Amino acid sequence of heavy chain of antibody 3
QVQLVESGGGLVKPGGSLRLSCAASGFTFSDYYMSWIRQAPGKGLEWVSYISISGTTRYYADSVKGRFTISRDNAKNSLSLQMNSLRAEDTAVYYCARGPELLSQNYYYYYGMDVWGQGTTVTVSLASTKGPSVFPLAPSSKSTSGGTAALGCLVKDYFPEPVTVSWNSGALTSGVHTFPAVLQSSGLYSLSSVVTVPSSSLGTQTYICNVNHKPSNTKVDKKVEPKSCDKTHTCPPCPAPELLGGPSVFLFPPKPKDTLMISRTPEVTCVVVDVSHEDPEVKFNWYVDGVEVHNAKTKPREEQYNSTYRVVSVLTVLHQDWLNGKEYKCKVSNKALPAPIEKTISKAKGQPREPQVYTLPPSRDELTKNQVSLTCLVKGFYPSDIAVEWESNGQPENNYKTTPPVLDSDGSFFLYSKLTVDKSRWQQGNVFSCSVMHEALHNHYTQKSLSLSPGK

SEQ ID NO: 45 - DNA, 660 bp, synthetic construct
  misc_feature 1..660: note = Nucleotide sequence of the light chain of antibody 3
  source 1..660: mol_type = other DNA
gacatcgagatgacccagagccccgacagcctggccgtgagcctgggcgagagagccaccatcaactgcaagagcagcgagaccctgctgtacagaagcaacaacaagaattacctggcctggtaccagcagaagcccggccagccccctaggctgctgctgtactgggccagcacacgggagtccggcgtgcctgacaggatctccggctccggctccggcaccgatttcaccctgaccatctcctccctgcaggccgaggatgtggccgtgtactactgccagcagtactacaccacaccacggacattcggccagggcacaaaggtggagatcaagcgtacggtggctgcaccatctgtcttcatcttcccgccatctgatgagcagttgaaatctggaactgcctctgttgtgtgcctgctgaataacttctatcccagagaggccaaagtacagtggaaggtggataacgccctccaatcgggtaactcccaggagagtgtcacagagcaggacagcaaggacagcacctacagcctcagcagcaccctgacgctgagcaaagcagactacgagaaacacaaagtctacgcctgcgaagtcacccatcagggcctgagctcgcccgtcacaaagagcttcaacaggggagagtgt

SEQ ID NO: 46 - protein, 220 aa, synthetic construct
  REGION 1..220: note = Amino acid sequence of the light chain of antibody 3
DIEMTQSPDSLAVSLGERATINCKSSETLLYRSNNKNYLAWYQQKPGQPPRLLLYWASTRESGVPDRISGSGSGTDFTLTISSLQAEDVAVYYCQQYYTTPRTFGQGTKVEIKRTVAAPSVFIFPPSDEQLKSGTASVVCLLNNFYPREAKVQWKVDNALQSGNSQESVTEQDSKDSTYSLSSTLTLSKADYEKHKVYACEVTHQGLSSPVTKSFNRGEC

SEQ ID NO: 47 - DNA, 1350 bp, synthetic construct
  misc_feature 1..1350: note = Nucleotide sequence of the heavy chain of antibody 4
  source 1..1350: mol_type = other DNA
gaggtgcagctggttgaatctggcggcggattggttcagcctggcggatctctgagactgtcttgtgctgcctctggcggcttcatcacctctcaccattgggtccgacaggcccctggcaaaggactggaatgggttgccagactgcaccacaccggcaccacacactacgccgattctgtgaagggcagattcaccatctccgccgacacctccaagaacaccgcctacctgcagatgaactccctgagagccgaggacaccgccgtgtactactgtgtgcgcgaggactcctcttcttggcaccctggcagatatatccagctgtggggccagggcacactggtcacagtttcttccgcctccaccaagggacccagcgttttccctctggctccatcctccaagtctacctccggtggaacagctgctctgggctgcctggtcaaggactactttcctgagcctgtgaccgtgtcctggaactctggcgctctgacatctggcgtgcacacctttccagcagtgctgcagtcctccggcctgtactctctgtcctctgtcgtgaccgtgccttccagctctctgggaacccagacctacatctgcaatgtgaaccacaagccttccaacaccaaggtggacaagaaggtggaacccaagtcctgcgacaagacccacacctgtcctccatgtcctgctccagaactgctcggcggaccttccgtgtttctgttccctccaaagcctaaggacaccctgatgatctctcggacccctgaagtgacctgcgtggtggtggatgtgtctcacgaggatcccgaagtgaagttcaattggtacgtggacggcgtggaagtgcacaacgccaagaccaagcctagagaggaacagtacaactccacctacagagtggtgtccgtgctgaccgtgctgcaccaggattggctgaacggcaaagagtacaagtgcaaggtgtccaacaaggccctgcctgctcctatcgaaaagaccatctccaaggccaagggccagcctagggaaccccaggtttacaccctgcctccaagccgggaagagatgaccaagaaccaggtgtccctgacctgcctcgtgaagggcttctacccttccgatatcgccgtggaatgggagagcaatggccagcctgagaacaactacaagacaacccctcctgtgctggactccgacggctcattcttcctgtactccaagctgacagtggacaagtccagatggcagcagggcaacgtgttctcctgctccgtgatgcacgaggccctgcacaatcactacacccagaagtccctgtctctgtcccctggctaa

SEQ ID NO: 48 - protein, 449 aa, synthetic construct
  REGION 1..449: note = Amino acid sequence of the heavy chain of antibody 4
EVQLVESGGGLVQPGGSLRLSCAASGGFITSHHWVRQAPGKGLEWVARLHHTGTTHYADSVKGRFTISADTSKNTAYLQMNSLRAEDTAVYYCVREDSSSWHPGRYIQLWGQGTLVTVSSASTKGPSVFPLAPSSKSTSGGTAALGCLVKDYFPEPVTVSWNSGALTSGVHTFPAVLQSSGLYSLSSVVTVPSSSLGTQTYICNVNHKPSNTKVDKKVEPKSCDKTHTCPPCPAPELLGGPSVFLFPPKPKDTLMISRTPEVTCVVVDVSHEDPEVKFNWYVDGVEVHNAKTKPREEQYNSTYRVVSVLTVLHQDWLNGKEYKCKVSNKALPAPIEKTISKAKGQPREPQVYTLPPSREEMTKNQVSLTCLVKGFYPSDIAVEWESNGQPENNYKTTPPVLDSDGSFFLYSKLTVDKSRWQQGNVFSCSVMHEALHNHYTQKSLSLSPG

SEQ ID NO: 49 - DNA, 660 bp, synthetic construct
  misc_feature 1..660: note = Nucleotide sequence of the light chain of antibody 4
  source 1..660: mol_type = other DNA
gacatccagatgacccagtctccatcctctctgtccgcctctgtgggcgacagagtgaccatctcctgccggtcatctcagtccctgctgcagaacaaccggtacaacagattcgactggtatcagcagaagcccggcaaggcccctaagctgctgatctacctgggctccaatagagcctctggcgtgccctctagattctccggctctagatctggcaccgactttaccctgacaatctccagcctgcagcctgaggacttcgccacctactactgcatgcacgccctggaacctccatacacctttggccagggcaccaaggtggaaatcaagcggacagtggccgctccttccgtgttcatcttcccaccttccgacgagcagctgaagtccggcacagcttctgtcgtgtgcctgctgaacaacttctaccctcgggaagccaaggtgcagtggaaggtggacaatgccctgcagtccggcaactcccaagagtctgtgaccgagcaggactccaaggacagcacctacagcctgtcctccacactgaccctgtccaaggccgactacgagaagcacaaggtgtacgcctgcgaagtgacccatcagggcctgtctagccctgtgaccaagtctttcaaccggggcgagtgctga

SEQ ID NO: 50 - protein, 219 aa, synthetic construct
  REGION 1..219: note = Amino acid sequence of the light chain of antibody 4
DIQMTQSPSSLSASVGDRVTISCRSSQSLLQNNRYNRFDWYQQKPGKAPKLLIYLGSNRASGVPSRFSGSRSGTDFTLTISSLQPEDFATYYCMHALEPPYTFGQGTKVEIKRTVAAPSVFIFPPSDEQLKSGTASVVCLLNNFYPREAKVQWKVDNALQSGNSQESVTEQDSKDSTYSLSSTLTLSKADYEKHKVYACEVTHQGLSSPVTKSFNRGEC